European Patent Application EP 4 269 597 A1, published November 1, 2023. Title: L-Histidine Export Protein and Method of Producing L-Histidine Using the Same. Applicant: CJ CheilJedang Corporation. The sequence listing filed with the application follows.

SEQUENCE LISTING (69 sequences)

SEQ ID NO: 1 - protein, 314 aa, Artificial Sequence
  Haq protein
MKSKNATLVGLSAVVLWSAIVGLIRGVSEHLGATGGAAAIYTVASLILLVSVGFPRLASFPRRYLLWGSVLFVAYELCLSLSIGYAHTGRQAIEVGMVNYLWPTFTLVAAILFGGQRATLLVVPGFILSMLGICWVLGGDQGLDPSGMLANIRDNPLSYGLAFIGALIWAAYCTVTTRIAQGQNGVTPFFMLVALALWVKVLLGGHVAELSFSVPALVYLVLAAAAMGLGYAAWNVGILHGNVTVLAGASYFIPVFSSALSALLLRAPLPTSFWVGAALVCAGSILCWRATRSLDLSKEPAARAARPEGPPQNQ

SEQ ID NO: 2 - DNA, 945 bp, Artificial Sequence
  haq gene
atgaagagcaagaacgcaaccctggtcggattgagcgcggtggtactgtggagtgccatcgtgggcctgatccgtggcgtgagcgagcatctcggagccaccggcggggcggcggccatttacacggtggcttcgctgatcctgctggtgtcggtgggattcccgcgcctggcgagtttcccgcgcaggtatctgctatggggcagcgtgctgttcgtggcttatgaattgtgcctgtcgctctcgatcggttatgcccataccggccgccaggccatcgaagtcggcatggtcaattacctctggccgaccttcaccctggtggcggccatcctcttcggaggccagcgcgccacgctgctggtggtgccaggcttcatcctttccatgctgggcatctgctgggtgctcgggggcgaccaggggctggatccttccggcatgctggccaatatccgtgacaatccgctgagctacggcctggccttcatcggggccttgatctgggcggcctactgcaccgtgactacccgcatcgcccaaggccagaacggggtgacgcctttcttcatgctggtggcattggcattgtgggtgaaggtgctgctgggcgggcatgtggctgaactatccttcagtgtgcccgcactggtctacctggtgctggctgcggcggcgatggggctgggctatgcggcctggaacgtgggcatcctgcatggcaatgtgacagtgctggccggtgcctcgtatttcatcccggtcttttcttcggccttgtcggccttgctgctacgtgcgccgctgcccacctcgttctgggtgggcgctgcgctggtgtgcgccgggtcgatcctgtgctggcgggctacccgcagcctggatttgtcaaaagaacctgcagcgcgggcggcacgtcccgaaggcccacctcagaaccaatag

SEQ ID NO: 3 - protein, 312 aa, Artificial Sequence
  Cpi protein
MQSTRKATLIGLIAILLWSSIVGLIRGVSESLGATGGAAMMYSVASVLLMLTVGFVRLREFPRRYLVWGSILFVSYELCLSLSIGYSHSGRQAIEVGMVNYLWPSFTMLCAIAFNKQKANVLIVPGFLIAILGICLVLGGEQGLDVAGMVANVRDNPLSYGLALAGALIWAAYCTVTNRIAGGNNGVTLFFMLTAMALWIKYFTGDHAPMAFTYHAVIYLALAASAMGFGYPAWNVGILHGNVTVLAGASYFIPVISAALAGLLLHIPLSLAFWKGASLVCAGSVLCWLATRARKVAATPDRAPVRDRVWKQ

SEQ ID NO: 4 - DNA, 939 bp, Artificial Sequence
  cpi gene
atgcaaagcacgcgtaaggccacgttgatcgggctcattgcgatcctgttgtggagttccatcgtcggcctgatccgcggcgtcagtgaaagcctcggcgcgaccggtggcgccgccatgatgtactcggttgcctccgtcctgcttatgctgacggttggcttcgtgcgtctgcgcgaatttccgcggcgctatctggtctggggcagcatcctgttcgtctcctacgaactgtgcctgtcgctgtccatcggctattcgcacagcggcaggcaggcgatcgaggtggggatggtcaattacctctggccgtctttcaccatgttgtgcgccatcgccttcaacaagcagaaggcgaacgttctgatcgtgccgggcttcctgattgcgatcctgggtatctgcctggtgctgggcggcgagcagggtctggatgttgcaggcatggtggccaatgtcagggacaatccgctcagctacggcctcgctttagcgggcgcgctgatctgggcggcctattgcaccgtgaccaacaggattgccggcggcaacaacggcgtcacgctgtttttcatgctcaccgcaatggcgctgtggatcaagtacttcaccggcgaccatgcgccgatggctttcacataccacgccgtcatctacctggcactggcagcgtcggcgatgggcttcggctacccggcgtggaacgtgggcatcctgcacggcaacgtaacggtgcttgccggcgcgtcgtatttcatccctgtgatttcagccgcactggctggcttgctcttgcatataccgctttcgctggcgttctggaaaggcgcgtcgctggtatgcgcggggtccgtgctgtgctggttggcgacgcgcgcgcgcaaggtggctgcaacgcccgaccgtgctccggtccgcgaccgtgtctggaagcaatga

SEQ ID NO: 5 - protein, 293 aa, Artificial Sequence
  Kcr protein
MDKKRATLIGFSAIILWSTMVGLIRGVSEGLGPVGGAAMIYSLSGLLLIFTVGFPQLRQIPPRYLLVGSLFFVSYEMCLALSLGYAGTRQQAIEVGMVNYLWPSLTILFAIIFNGQKTTWLVIPGLLLSIVGVTWVLGGEHGLDLAEIRSNVISSPLSYILAFVGAFIWAAYCTVTAKYAKGKNGITLFVLFTALALWVKFLMSEQPPMIFSWPVVIKLVTCALALGFAYAAWNVGILHGNVSLLAAASYFTPVLSSALAAFLLSAALSWSFWQGAAMVCGGSLLCWYATRRP

SEQ ID NO: 6 - DNA, 371 bp, Artificial Sequence
  kcr gene
atggataagaaaagagcgacgctcattggatttagcgccattattttgtggagtacgatggtgggtctgattcgcggcgtaagcgaagggctcggcccggtgggcggagccgcaatgatttacagcctcagcggcctgctgctgatttttaccgttggcttcccacaattgcgccaaattccaccgcgctatttgctggtaggtagcctgttttttgtcagctacgaaatgtgcctcgcgctctcattaggctatgccggcactcgccaacaggccatcgaagtcggcatggtgaattatctctggcctagcctgacgattttatttgcgattatctttaatggtcaaaaaaccacctggctggttatccc

SEQ ID NO: 7 - protein, 238 aa, Artificial Sequence
  Cst protein
MSTLSILIAGFALGLSLIVAIGPQNALLIKQGIKREHVWVVIAICAVSDIILISGGTAGVGYLVETFPTALVVLKYLGAIYLAYFTYLCFRDALRDKVETLSPAQIEPNKTQQIDAFDGGDLGGSSVDTRRRTTRLRQQVRQSTWVKPALATLAICWLNPAAYVDVLVMIGGLANQYGETGRWFFAAGAIAASMLWFPSVGLAAAKFSHVLSRPAVWRGINFGIGCIMALLTIKLLLT

SEQ ID NO: 8 - DNA, 717 bp, Artificial Sequence
  cst gene
atgtcaacgctgtctatcctcatcgccggtttcgcactagggctctcacttatcgtagcgattggcccgcaaaatgctctgctgatcaaacagggcattaaacgcgagcacgtgtgggtagtcattgcgatttgcgcggtgtccgacattattttgattagcggtggcaccgcgggggtgggctatctggtggagactttcccgaccgcactggtggtgctgaagtatctgggcgcgatttatctggcttactttacttatctgtgctttcgcgatgcgttgcgcgacaaggttgaaactctctcccctgcgcagatcgagccgaataagacgcagcagatcgatgcattcgatggcggcgacttgggcggttcttctgttgatacccggcggcgcaccacgcgtctgcgccagcaagtacgccaatcgacctgggtgaagccagctcttgcgaccttggcgatttgctggctgaacccggcagcttatgtcgatgtgctggtaatgattggcggacttgccaaccaatacggcgaaaccggccgatggttttttgctgccggtgccattgcagcgagcatgctgtggtttcccagcgttggtcttgctgccgcgaagttctcgcacgtactttcgcgccctgcggtatggcgcggcatcaacttcggcattggctgcatcatggcgctgctgaccattaagctgctgttgacctag

SEQ ID NO: 9 - protein, 242 aa, Artificial Sequence
  LsaF protein
MSPSHDPLPRRAGAAAGLRDSLGVGLGIFPLGIALGILVIQAGLPWWLAPALSIGIFAGSVELLLVSMLAAATPLVTIAATVFAVNFRHVFYAFSFPLSRVRPGLPRAYSIYAMIDEAYATYVLMDPDRLSSARMVTGQLAMQLYWVLGGFVGIMIANVLPAPIEGFEFALVALFVVMSMDAIRGKRELPSALLACLAVTVAILVAGDNALLVALALYSGLLGLRYFLTKRTTDTAEEGERA

SEQ ID NO: 10 - protein, 140 aa, Artificial Sequence
  LsaE protein
MRCWSRLRCTPGYWGCAISSPSEPRTLRRRASVPSTEYLIAGVVVAGLITLALRALPFAALKPLRKSKLVQALGRWMPAGILVILAVVVLRDQLISQQGRVWPVLVATAITALAHLLSKRRALVSIAAGTACYVLLLNFF

SEQ ID NO: 11 - DNA, 1048 bp, Artificial Sequence
  lsa gene
atgtctccgtcacacgatcctttaccgcgccgcgcgggcgccgcggccggccttcgagattctctcggggtcggcctcggcattttccccttgggcattgccctcggaattcttgtcattcaggcgggacttccctggtggctcgccccggccctctcgattggtatcttcgcgggatctgtcgagctgctcctggtcagcatgctcgccgccgcgactccgctcgtgacgatcgccgcgaccgtgttcgccgtgaactttcggcacgtattctacgcgttctcgtttccgctttcgcgggtgcgaccgggtctaccccgggcgtactccatctacgcaatgatcgacgaggcctacgccacctatgtgctgatggatccggatcgcctgagctcagcccgcatggtaaccggccagctcgcgatgcagctctattgggtgctcggcggcttcgtcggcatcatgattgcgaacgtgctccctgcccccattgagggctttgagtttgcactcgtggcgctcttcgtggtgatgtcgatggatgcgattcgcggcaagcgcgagctcccatcggccttgctggcttgcctcgctgtcacggttgcaatactggtcgctggcgacaatgcgctgctggtcgcgcttgcgctgtactccgggctactggggctgcgctatttcctcaccaagcgaaccacggacactgcggaggagggcgagcgtgcctagcaccgaatatctaatcgcgggcgtcgtcgtcgcgggcctcatcaccctggcgctgcgcgcactcccgtttgcggcgctcaaaccgctgcgcaaatctaagctcgtgcaggcgctcgggcgctggatgcccgctggcatcctcgttatcctcgccgtcgtcgtactgcgcgatcagctcatatcgcagcagggccgggtgtggccggtgctcgtcgcgaccgcgatcacggccctcgctcacttgctctcaaagcgacgcgcgctcgtgagcatcgcggctggcaccgcctgctacgtgctgctgctcaactttttctag

SEQ ID NO: 12 - protein, 251 aa, Artificial Sequence
  DvaF protein
MSVEAQPGANDRPYSVRHEITQGALLILPAGLGMIPIGIAFGLLVVQSGLPWWMAPALSFFAYAGSLELLLITLITSLTPLVTIAAASFFVNFRHVFYAFNFPLKVVTNPFLKFYAMYSLTDEIFAVTVANPKGWTQPRVISAGAVLQICWVGGGLMGVLLSSFIPFQIRGLSFALCALFITLTLDACRTKQEIPSLLLGAAAFGFALLLLPSQPIFAAMIGFVATLAARYTIAVRLTRPLPAEMESDDAA

SEQ ID NO: 13 - protein, 111 aa, Artificial Sequence
  DvaE protein
MQLDIPFWYLASVLLIAFAVTFTLRALPFAILEPLRKSQFVRVMAVWMPAGILVILALATFKSTLAEEPGGLVHLLIASGVTIAVHLFGGRRTLVSVAAGTLAFVLLVNFF

SEQ ID NO: 14 - DNA, 1081 bp, Artificial Sequence
  dvaFE gene
atgagcgttgaggcgcagcctggcgcaaacgaccgaccctatagcgtgcgccacgagatcacgcagggcgcactcctgattctccccgcagggctcggaatgattccgatcggcattgccttcggcctgcttgtggtgcaatcggggctcccgtggtggatggcacccgccctttcgttcttcgcgtacgcgggctcactcgagcttctgctcatcacgctcatcacgtcgcttacgccgcttgtaacgatcgctgcggcatcgttcttcgtgaacttccgccacgtgttctacgcgtttaatttcccgctcaaggtcgtcacgaacccgttcttgaagttctacgcgatgtactccctcaccgacgagatcttcgcggtaacggttgccaatccaaaggggtggacgcagccgcgcgtgatctcggcaggggccgtactccagatctgctgggtgggtggcggcctcatgggggtactgctctcgagcttcatccccttccagatccgcggcctgagtttcgcgctgtgcgccctgttcatcacgctgaccctcgatgcgtgccgcacgaaacaggagatcccgtcacttctcctcggtgctgccgccttcggtttcgcgctccttttgctcccgagccagccgatcttcgccgcgatgattggcttcgtggcgaccctcgccgcgcgctacacgatcgccgtgcgcctcacgaggccactcccggcagagatggagagcgacgatgcagcttgacatccccttctggtatctcgcctcggttctcctcatcgccttcgccgtgaccttcacgctgcgcgcgctcccgttcgcgattctcgaaccactgcgcaaatcgcaattcgtgcgcgtcatggccgtgtggatgcccgcgggcatcctcgtgatcctcgcgctcgcgacctttaagagcaccctcgccgaggaacccggtggtctcgttcacctgctgatcgcctcaggagtcacgattgccgtgcacctcttcggtggtcgccgcaccctcgtgagcgtcgccgcgggcaccctcgccttcgtgctgctcgtgaactttttctaa

SEQ ID NO: 15 - DNA, 409 bp, Artificial Sequence
  PgapA
tctgagactttaatttgtggattcacgggggtgtaatgtagttcataattaaccccattcgggggagcagatcgtagtgcgaacgatttcaggttcgttccctgcaaaaactatttagcgcaagtgttggaaatgcccccgtttggggtcaatgtccatttttgaatgtgtctgtatgattttgcatctgctgcgaaatctttgtttccccgctaaagttgaggacaggttgacacggagttgactcgacgaattatccaatgtgagtaggtttggtgcgtgagttggaaaaattcgccatactcgcccttgggttctgtcagctcaagaattcttgagtgaccgatgctctgattgacctaactgcttgacacattgcatttcctacaatctttagaggagacacaac

SEQ ID NO: 16 - DNA, 40 bp, Artificial Sequence
  Primer
gtacccggggatcctctagacaaagccgaagagaagttgg

SEQ ID NO: 17 - DNA, 30 bp, Artificial Sequence
  Primer
gcatagagtactcggcgcccataaatttca

SEQ ID NO: 18 - DNA, 30 bp, Artificial Sequence
  Primer
gcgccgagtactctatgccgagaagttgaa

SEQ ID NO: 19 - DNA, 40 bp, Artificial Sequence
  Primer
gcctgcaggtcgactctagactgggcatcacactattttt

SEQ ID NO: 20 - DNA, 531 bp, Artificial Sequence
  del-N2131L
gtacccggggatcctctagacaaagccgaagagaagttggcttgacggacccgaaattccagctgattttgacgatcctgatgcacccggcaggtggcctggcgaaaagttggggcttcctcaagaaggggccggctctctgtcctcagtggctcgtcgtatcggcggggtctgcgtggactggggtgtttcctgggttattgctattgtgctgtccaatttcacggatgtgctgggcgatgtagcgacatccacgctcattattttcgtgatcctgggttggcttaccggttggatctttgctcgcaccccaggtcatgccgtgtttggcatgggccttgcgcgtgtggatgcagaggaacgtgtgggctggtggcgtgcgctggttcgcccactgctgacgatcttgattctgcctgccgtgatggtggatgctgacggccgtgggctccacgacaaggcaacgggaactgcagttatccgcgggtaatttgtcttgagtgaaatttatgggcgccgagtactctatgc

SEQ ID NO: 21 - DNA, 555 bp, Artificial Sequence
  del-N2131R
gcgccgagtactctatgccgagaagttgaacagcaatcttgcagcaactcctcagtattcacaccagccccaatggacacaaaaacatcagccccagaatcgcccctaagggcctcaaatacacgatctggaccaactagtcatcgggaaaacccaaccccttaaatcgccttctgcgcttaaggggtcaatgctagataagtaggaacaacaacgtttgggcggccaggatctttgcgatcatcgccagcggatacacagaggtataacccatggcagggagctcgttgcgggaggcatctgacacataactcagcacagcagggtgggtttgcgtaccggcgaggatgccagcggtttcaccgaaggggattttcatcagtttgtggccaacgaacagcaccgtgatggagatgaacaaagtgagcagcgcaccgaagccgatgatggtgagtgattgggggtcgctgatcgctgatcgaaatcctgcgcccgctgaggtaccgatggcagccaaaaatagtgtgatgcccagtctagagtcgacctgcaggc

SEQ ID NO: 22 - DNA, 30 bp, Artificial Sequence
  Primer
aggagacacaacatgaagagcaagaacgca

SEQ ID NO: 23 - DNA, 40 bp, Artificial Sequence
  Primer
tcaacttctcggcatagagtctattggttctgaggtgggc

SEQ ID NO: 24 - DNA, 40 bp, Artificial Sequence
  Primer
gaaatttatgggcgccgagttctgagactttaatttgtgg

SEQ ID NO: 25 - DNA, 30 bp, Artificial Sequence
  Primer
cttgctcttcatgttgtgtctcctctaaag

SEQ ID NO: 26 - DNA, 30 bp, Artificial Sequence
  Primer
aggagacacaacatgcaaagcacgcgtaag

SEQ ID NO: 27 - DNA, 40 bp, Artificial Sequence
  Primer
tcaacttctcggcatagagttcattgcttccagacacggt

SEQ ID NO: 28 - DNA, 30 bp, Artificial Sequence
  Primer
cgtgctttgcatgttgtgtctcctctaaag

SEQ ID NO: 29 - DNA, 30 bp, Artificial Sequence
  Primer
aggagacacaacatggataagaaaagagcg

SEQ ID NO: 30 - DNA, 40 bp, Artificial Sequence
  Primer
tcaacttctcggcatagagtttagggacggcgggtggcgt

SEQ ID NO: 31 - DNA, 30 bp, Artificial Sequence
  Primer
tttcttatccatgttgtgtctcctctaaag

SEQ ID NO: 32 - DNA, 30 bp, Artificial Sequence
  Primer
aggagacacaacatgtcaacgctgtctatc

SEQ ID NO: 33 - DNA, 40 bp, Artificial Sequence
  Primer
tcaacttctcggcatagagtctaggtcaacagcagcttaa

SEQ ID NO: 34 - DNA, 30 bp, Artificial Sequence
  Primer
cagcgttgacatgttgtgtctcctctaaag

SEQ ID NO: 35 - DNA, 30 bp, Artificial Sequence
  Primer
aggagacacaacatgtctccgtcacacgat

SEQ ID NO: 36 - DNA, 40 bp, Artificial Sequence
  Primer
tcaacttctcggcatagagtctagaaaaagttgagcagca

SEQ ID NO: 37 - DNA, 30 bp, Artificial Sequence
  Primer
tgacggagacatgttgtgtctcctctaaag

SEQ ID NO: 38 - DNA, 30 bp, Artificial Sequence
  Primer
aggagacacaacatgagcgttgaggcgcag

SEQ ID NO: 39 - DNA, 40 bp, Artificial Sequence
  Primer
tcaacttctcggcatagagtttagaaaaagttcacgagca

SEQ ID NO: 40 - DNA, 30 bp, Artificial Sequence
  Primer
ctcaacgctcatgttgtgtctcctctaaag

SEQ ID NO: 41 - protein, 251 aa, Artificial Sequence
  HmaF protein
MSVAAQPSAHEHPYSVRHEITQGALLILPAGLGMIPIGIAFGLLVVQSGLPWWMAPALSFFAYAGSLELLLITLITSLTPLVTIAAASFFVNFRHVFYAFNFPLKVVKNPFLKFYAMYSLTDEIFAVTVAHPKGWTQPRVISAGAVLQICWVGGGLMGVLLSSFIPFQIRGLSFALCALFITLTLDACRTKQELPSLVLGAAAFGLALLLMPGQPIFAAMIGFVATLAARYTIAVRLTRPLPAEMEGDDAA

SEQ ID NO: 42 - protein, 111 aa, Artificial Sequence
  HmaE protein
MQLDIPFWYLASVLLIAFAVTFTLRALPFAILEPLRKSQFVRVMAVWMPAGILVILALATFKSTLAEEPGSVIHLLIASAVTIAVHLLFGRRTLVSVAAGTLAFVLLVNFF

SEQ ID NO: 43 - DNA, 1081 bp, Artificial Sequence
  hmaFE gene
atgagcgttgcggcgcagcctagcgcacatgagcatccctattcggtgcgccatgaaatcacgcagggggcgctcttgattctccccgcgggcctcggcatgatcccgattggcatcgcttttggccttcttgttgtgcagtccggacttccgtggtggatggcacccgccctctcattcttcgcgtacgcgggctcgctcgagcttttgctcatcacactcatcacatcgctcacgccgctcgtgacgatcgctgcggcatcgttcttcgtgaacttccgccacgtgttttacgcgttcaacttcccgctcaaggtcgtgaagaacccgtttttgaagttctacgcgatgtactcgcttaccgacgagatcttcgcggtgacggtcgcgcacccgaaggggtggacgcagccacgcgtcatctccgcgggcgccgtactccagatctgctgggtgggaggcggcctcatgggcgtgctcctctcgagtttcattcccttccagatccgcggtttgagcttcgccctgtgcgcgcttttcatcaccctgactctcgatgcgtgccgcacgaagcaagaacttccgtcgctagttctcggcgccgcggccttcggtctcgccctgctcctcatgcccgggcagccgatctttgccgcgatgatcggcttcgttgcaacgctcgccgcgcggtacacgatcgccgtgcgccttacgaggccgctaccggcggaaatggagggcgacgatgcagcttgacatccccttctggtaccttgcctcggttctcctcattgccttcgccgtcacctttacgctgcgcgcgctcccgttcgcgatcctcgaaccgctgcgcaaatcccagttcgtgcgcgtcatggccgtgtggatgcccgcgggcatcctcgtcattctcgcgctcgcgaccttcaaaagcaccctcgctgaggaacccggcagcgtcattcatttgctcattgcctcggccgtcacgatcgctgtgcatcttctctttgggcgccgaaccctcgtgagtgtcgccgcgggtaccctcgccttcgtgctcctcgtgaacttcttctaa

SEQ ID NO: 44 - protein, 251 aa, Artificial Sequence
  MabF protien
MSVEAQPGAHERPYSVRHEITQGALLILPAGLGMIPIGIAFGLLVVQSGLPWWMAPALSFFAYAGSLELLLITLITSLTPLVTIAAASFFVNFRHVFYAFNFPLKVVKNPFLKFYAMYSLTDEIFAVTVANPKGWTQPRVISAGAVLQICWVGGGLMGVLLSSFIPFQIRGLSFALCALFITLTLDACRTKQEIPSLLLGAAAFGLALLLLPSQPIFAAMIGFVATLAARYTIAVRLTRPLPAEMESDDAA

SEQ ID NO: 45 - protein, 111 aa, Artificial Sequence
  MabE protein
MQLDIPFWYLASVLLIAFAVTFTLRALPFAILEPLRKSQFVRVMAVWMPAGILVILALATFKSTLAEEPGGLVHLLIASAVTIAVHLFGGRRTLVSVAAGTLAFVLLVNFF

SEQ ID NO: 46 - DNA, 1081 bp, Artificial Sequence
  mabFE gene
atgagcgttgaggcgcagcctggcgcacacgagcgaccctactcggtgcgccacgaaatcacgcagggcgcgctcctgattctccccgcaggtctcggcatgatcccgatcggtatcgccttcggcctgcttgtggtgcagtcggggctcccgtggtggatggcgcccgccctctcgtttttcgcgtacgcgggctcactcgagcttctgctcatcacgctcatcacgtcgcttaccccactggtgacgatcgcggcggcatcgttcttcgtgaacttccgccacgtgttctacgcgttcaactttccactcaaggtcgtgaagaacccgtttttgaagttctacgcgatgtattcgctgaccgacgaaatcttcgcggtcacggtcgcgaacccaaaggggtggacccagccgcgcgtgatctcggcaggggccgtactccagatctgctgggtgggtggcggcctcatgggggtactgctctcgagcttcatccccttccagatccgcggcctgagtttcgcgctgtgcgccctgttcatcacgctgaccctcgatgcgtgccgcacaaaacaggagatcccgtcacttctcctcggcgctgccgccttcggcctcgcgcttcttttgctcccgagccagccgatcttcgcggcgatgattggcttcgttgcgaccctcgcggctcgctacacgatcgccgtacgcctcacgaggccactcccggcagagatggagagcgacgatgcagcttgacatccccttctggtacctcgcctcggttctcctcatcgccttcgccgttacttttacgctgcgcgcgctcccgttcgcgatcctcgaaccactgcgcaaatcgcaattcgtgcgcgtcatggccgtgtggatgcccgcgggcatcctcgtcattctggcgctcgcgaccttcaagagcaccctcgccgaggaacccggtggtctcgttcacctgctgatcgcctcagccgtcacgatcgccgtgcacctcttcggtggtcgccgaaccctcgtgagcgtcgccgcgggcaccctcgccttcgtgctgctcgtgaacttcttctaa

SEQ ID NO: 47 - DNA, 30 bp, Artificial Sequence
  Primer
aggagacacaacatgagcgttgcggcgcag

SEQ ID NO: 48 - DNA, 40 bp, Artificial Sequence
  Primer
tcaacttctcggcatagagtttagaagaagttcacgagga

SEQ ID NO: 49 - DNA, 30 bp, Artificial Sequence
  Primer
cgcaacgctcatgttgtgtctcctctaaag

SEQ ID NO: 50 - DNA, 30 bp, Artificial Sequence; identical to SEQ ID NO: 38
  Primer

SEQ ID NO: 51 - DNA, 40 bp, Artificial Sequence
  Primer
tcaacttctcggcatagagtttagaagaagttcacgagca

SEQ ID NO: 52 - DNA, 30 bp, Artificial Sequence; identical to SEQ ID NO: 40
  Primer

SEQ ID NO: 53 - DNA, 100 bp, Artificial Sequence
  PyccA
ttccagatcaaatgcgtaaagatgggtaaaacttctgggtgcccttacgcattatcattatgctgcttaattaattacatctgtcatagagagtgactca

SEQ ID NO: 54 - DNA, 30 bp, Artificial Sequence
  Primer
gagagtgactcaatgagcgttgaggcgcag

SEQ ID NO: 55 - DNA, 40 bp, Artificial Sequence
  Primer
cgggtaccgagctcgaattcttagaaaaagttcacgagca

SEQ ID NO: 56 - DNA, 40 bp, Artificial Sequence
  Primer
actcactatagggcgaattcttccagatcaaatgcgtaaa

SEQ ID NO: 57 - DNA, 30 bp, Artificial Sequence
  Primer
ctcaacgctcattgagtcactctctatgac

SEQ ID NO: 58 - DNA, 30 bp, Artificial Sequence
  Primer
gagagtgactcaatgagcgttgcggcgcag

SEQ ID NO: 59 - DNA, 40 bp, Artificial Sequence
  Primer
cgggtaccgagctcgaattcttagaagaagttcacgagga

SEQ ID NO: 60 - DNA, 30 bp, Artificial Sequence
  Primer
cgcaacgctcattgagtcactctctatgac

SEQ ID NO: 61 - DNA, 30 bp, Artificial Sequence; identical to SEQ ID NO: 54
  Primer

SEQ ID NO: 62 - DNA, 40 bp, Artificial Sequence
  Primer
cgggtaccgagctcgaattcttagaagaagttcacgagca

SEQ ID NO: 63 - DNA, 30 bp, Artificial Sequence; identical to SEQ ID NO: 57
  Primer

SEQ ID NO: 64 - DNA, 756 bp, Artificial Sequence
  dvaF gene
atgagcgttgaggcgcagcctggcgcaaacgaccgaccctatagcgtgcgccacgagatcacgcagggcgcactcctgattctccccgcagggctcggaatgattccgatcggcattgccttcggcctgcttgtggtgcaatcggggctcccgtggtggatggcacccgccctttcgttcttcgcgtacgcgggctcactcgagcttctgctcatcacgctcatcacgtcgcttacgccgcttgtaacgatcgctgcggcatcgttcttcgtgaacttccgccacgtgttctacgcgtttaatttcccgctcaaggtcgtcacgaacccgttcttgaagttctacgcgatgtactccctcaccgacgagatcttcgcggtaacggttgccaatccaaaggggtggacgcagccgcgcgtgatctcggcaggggccgtactccagatctgctgggtgggtggcggcctcatgggggtactgctctcgagcttcatccccttccagatccgcggcctgagtttcgcgctgtgcgccctgttcatcacgctgaccctcgatgcgtgccgcacgaaacaggagatcccgtcacttctcctcggtgctgccgccttcggtttcgcgctccttttgctcccgagccagccgatcttcgccgcgatgattggcttcgtggcgaccctcgccgcgcgctacacgatcgccgtgcgcctcacgaggccactcccggcagagatggagagcgacgatgcagcttga

SEQ ID NO: 65 - DNA, 335 bp, Artificial Sequence
  dvaE gene
atgcagcttgacatccccttctggtatctcgcctcggttctcctcatcgccttcgccgtgaccttcacgctgcgcgcgctcccgttcgcgattctcgaaccactgcgcaaatcgcaattcgtgcgcgtcatggccgtgtggatgcccgcgggcatcctcgtgatcctcgcgctcgcgacctttaagagcaccctcgccgaggaacccggtggtctcgttcacctgctgatcgcctcaggagtcacgattgccgtgcacctcttcggtggtcgccgcaccctcgtgagcgtcgccgcgggcaccctcgccttcgtgctgctcgtgaactttttcta

SEQ ID NO: 66 - DNA, 756 bp, Artificial Sequence
  hmaF gene
atgagcgttgcggcgcagcctagcgcacatgagcatccctattcggtgcgccatgaaatcacgcagggggcgctcttgattctccccgcgggcctcggcatgatcccgattggcatcgcttttggccttcttgttgtgcagtccggacttccgtggtggatggcacccgccctctcattcttcgcgtacgcgggctcgctcgagcttttgctcatcacactcatcacatcgctcacgccgctcgtgacgatcgctgcggcatcgttcttcgtgaacttccgccacgtgttttacgcgttcaacttcccgctcaaggtcgtgaagaacccgtttttgaagttctacgcgatgtactcgcttaccgacgagatcttcgcggtgacggtcgcgcacccgaaggggtggacgcagccacgcgtcatctccgcgggcgccgtactccagatctgctgggtgggaggcggcctcatgggcgtgctcctctcgagtttcattcccttccagatccgcggtttgagcttcgccctgtgcgcgcttttcatcaccctgactctcgatgcgtgccgcacgaagcaagaacttccgtcgctagttctcggcgccgcggccttcggtctcgccctgctcctcatgcccgggcagccgatctttgccgcgatgatcggcttcgttgcaacgctcgccgcgcggtacacgatcgccgtgcgccttacgaggccgctaccggcggaaatggagggcgacgatgcagcttga

SEQ ID NO: 67 - DNA, 336 bp, Artificial Sequence
  hmaE gene
atgcagcttgacatccccttctggtaccttgcctcggttctcctcattgccttcgccgtcacctttacgctgcgcgcgctcccgttcgcgatcctcgaaccgctgcgcaaatcccagttcgtgcgcgtcatggccgtgtggatgcccgcgggcatcctcgtcattctcgcgctcgcgaccttcaaaagcaccctcgctgaggaacccggcagcgtcattcatttgctcattgcctcggccgtcacgatcgctgtgcatcttctctttgggcgccgaaccctcgtgagtgtcgccgcgggtaccctcgccttcgtgctcctcgtgaacttcttctaa

SEQ ID NO: 68 - DNA, 756 bp, Artificial Sequence
  mabF gene
atgagcgttgaggcgcagcctggcgcacacgagcgaccctactcggtgcgccacgaaatcacgcagggcgcgctcctgattctccccgcaggtctcggcatgatcccgatcggtatcgccttcggcctgcttgtggtgcagtcggggctcccgtggtggatggcgcccgccctctcgtttttcgcgtacgcgggctcactcgagcttctgctcatcacgctcatcacgtcgcttaccccactggtgacgatcgcggcggcatcgttcttcgtgaacttccgccacgtgttctacgcgttcaactttccactcaaggtcgtgaagaacccgtttttgaagttctacgcgatgtattcgctgaccgacgaaatcttcgcggtcacggtcgcgaacccaaaggggtggacccagccgcgcgtgatctcggcaggggccgtactccagatctgctgggtgggtggcggcctcatgggggtactgctctcgagcttcatccccttccagatccgcggcctgagtttcgcgctgtgcgccctgttcatcacgctgaccctcgatgcgtgccgcacaaaacaggagatcccgtcacttctcctcggcgctgccgccttcggcctcgcgcttcttttgctcccgagccagccgatcttcgcggcgatgattggcttcgttgcgaccctcgcggctcgctacacgatcgccgtacgcctcacgaggccactcccggcagagatggagagcgacgatgcagcttga

SEQ ID NO: 69 - DNA, 336 bp, Artificial Sequence
  mabE gene
atgcagcttgacatccccttctggtacctcgcctcggttctcctcatcgccttcgccgttacttttacgctgcgcgcgctcccgttcgcgatcctcgaaccactgcgcaaatcgcaattcgtgcgcgtcatggccgtgtggatgcccgcgggcatcctcgtcattctggcgctcgcgaccttcaagagcaccctcgccgaggaacccggtggtctcgttcacctgctgatcgcctcagccgtcacgatcgccgtgcacctcttcggtggtcgccgaaccctcgtgagcgtcgccgcgggcaccctcgccttcgtgctgctcgtgaacttcttctaa